European Patent Application EP 4 212 548 A1, published July 19, 2023. Title: ANTIVIRAL COMPOSITION FOR INFLUENZA A VIRUS. Applicant: NOVELGEN. The sequence listing filed with the application follows.

SEQUENCE LISTING (34 sequences)

SEQ ID NO: 1 - protein, 10 aa, Artificial Sequence
  VH CDR1
GYTFTSYVMH

SEQ ID NO: 2 - protein, 7 aa, Artificial Sequence
  VH CDR2
INPYNDG

SEQ ID NO: 3 - protein, 11 aa, Artificial Sequence
  VH CDR3
GAYKRGYAMDY

SEQ ID NO: 4 - protein, 17 aa, Artificial Sequence
  VL CDR1
KSSQSLFNSRTRKNYLA

SEQ ID NO: 5 - protein, 7 aa, Artificial Sequence
  VL CDR2
WASTRES

SEQ ID NO: 6 - protein, 9 aa, Artificial Sequence
  VL CDR3
KQSYYHMYT

SEQ ID NO: 7 - protein, 121 aa, Artificial Sequence
  VH
EVQLQQSGPELVKPGASVKMSCKASGYTFTSYVMHWVKQKPGQGLEWIGYINPYNDGTKYNEKFKGKATLTSDKSSSTAYMELSSLTSEDSAVYYCARGAYKRGYAMDYWGQGTSVTVSSR

SEQ ID NO: 8 - protein, 113 aa, Artificial Sequence
  VL
DLVMSQSPSSLAVSAGEKVTMSCKSSQSLFNSRTRKNYLAWYQQKPGQSPKLLIYWASTRESGVPDRFTGSGSGTDFTLTISSVQAEDLAVYYCKQSYYHMYTFGSGTKLEIK

SEQ ID NO: 9 - protein, 249 aa, Artificial Sequence
  3D8 scFv
EVQLQQSGPELVKPGASVKMSCKASGYTFTSYVMHWVKQKPGQGLEWIGYINPYNDGTKYNEKFKGKATLTSDKSSSTAYMELSSLTSEDSAVYYCARGAYKRGYAMDYWGQGTSVTVSSRGGGGSGGGGSGGGGSDLVMSQSPSSLAVSAGEKVTMSCKSSQSLFNSRTRKNYLAWYQQKPGQSPKLLIYWASTRESGVPDRFTGSGSGTDFTLTISSVQAEDLAVYYCKQSYYHMYTFGSGTKLEIK

SEQ ID NO: 10 - DNA, 747 bp, Artificial Sequence
  3D8 scFv gene
gaggtccagctgcagcagtctggacctgagctggtaaagcctggggcttcagtgaagatgtcctgcaaggcttctggatacacattcactagctatgttatgcactgggtgaagcagaagcctgggcagggccttgagtggattggatatattaatccttacaatgatggtactaagtacaatgagaagttcaaaggcaaggccacactgacttcagacaaatcctccagcacagcctacatggagctcagcagcctgacctctgaggactctgcggtctattactgtgcaagaggggcctataaaaggggatatgctatggactactggggtcaaggaacctcagtcaccgtctcctctagaggtgggggcggttcgggtggcgggggctcgggcgggggtggctcagatcttgtgatgtcacagtctccatcctccctggctgtgtcagcaggagagaaggtcactatgagctgcaaatccagtcagagtctgttcaacagtagaacccgaaagaactacttggcttggtaccagcagaaaccagggcagtctcctaaactgctgatctactgggcatccactagggaatctggggtccctgatcgcttcacaggcagtggatctgggacagatttcactctcaccatcagcagtgtgcaggctgaagacctggcagtttattactgcaagcaatcttattatcacatgtatacgttcggatcggggaccaagctggaaataaaa

SEQ ID NO: 11 - DNA, 22 bp, Artificial Sequence
  Hemagglutinin forward primer
gctaccatgcgaacaattcaac

SEQ ID NO: 12 - DNA, 22 bp, Artificial Sequence
  Hemagglutinin reverse primer
ctgcactgcaaagatccattag

SEQ ID NO: 13 - DNA, 21 bp, Artificial Sequence
  Neuramindase forward primer
ccattggatcaatctgtctgg

SEQ ID NO: 14 - DNA, 22 bp, Artificial Sequence
  Neuramindase reverse primer
tgtcaatggtgaatggcaactc

SEQ ID NO: 15 - DNA, 21 bp, Artificial Sequence
  Nucleoprotein forward primer
actgatggagaacgccagaat

SEQ ID NO: 16 - DNA, 21 bp, Artificial Sequence
  Nucleoprotein reverse primer
atgtcaaaggaaggcacgatc

SEQ ID NO: 17 - DNA, 21 bp, Artificial Sequence
  GAPDH (MDCK Cell Line) forward primer
aacatcatccctgcttccact

SEQ ID NO: 18 - DNA, 19 bp, Artificial Sequence
  GAPDH (MDCK Cell Line) reverse primer
ggcaggtcagatccacaac

SEQ ID NO: 19 - DNA, 20 bp, Artificial Sequence
  GAPDH (Mouse) forward primer
ggcattgctctcaatgacaa

SEQ ID NO: 20 - DNA, 20 bp, Artificial Sequence
  GAPDH (Mouse) reverse primer
tgtgagggagatgctcagtg

SEQ ID NO: 21 - DNA, 20 bp, Artificial Sequence
  Hemagglutinin (A/PuertoRico/8/1934 (H1N1)) forward primer
agtgcccaaaatacgtcagg

SEQ ID NO: 22 - DNA, 20 bp, Artificial Sequence
  Hemagglutinin (A/PuertoRico/8/1934 (H1N1)) reverse primer
cagtccatcccccttcaata

SEQ ID NO: 23 - DNA, 21 bp, Artificial Sequence
  Hemagglutinin (A/X-31 (H3N2)) forward primer
gaaaatggttgggagggaatg

SEQ ID NO: 24 - DNA, 21 bp, Artificial Sequence
  Hemagglutinin (A/X-31 (H3N2)) reverse primer
gatggctgcttgagtgctttt

SEQ ID NO: 25 - DNA, 19 bp, Artificial Sequence
  Hemagglutinin (A/California/07/2009(H1N1)) forward primer
ggaacgtgttacccaggag

SEQ ID NO: 26 - DNA, 20 bp, Artificial Sequence
  Hemagglutinin (A/California/07/2009(H1N1)) reverse primer
gctgccgttacacctttgtt

SEQ ID NO: 27 - DNA, 21 bp, Artificial Sequence
  Nucleoprotein (A/PuertoRico/8/1934 (H1N1)) forward primer
accaatcaacagagggcatct

SEQ ID NO: 28 - DNA, 21 bp, Artificial Sequence
  Nucleoprotein (A/PuertoRico/8/1934 (H1N1)) reverse primer
tgatttcggtcctcatgtcag

SEQ ID NO: 29 - DNA, 21 bp, Artificial Sequence
  Nucleoprotein (A/X-31 (H3N2)) forward primer
aaaatcatggcgtctcaaggc

SEQ ID NO: 30 - DNA, 21 bp, Artificial Sequence
  Nucleoprotein (A/X-31 (H3N2)) reverse primer
cggtgcacatttggatgtaga

SEQ ID NO: 31 - DNA, 20 bp, Artificial Sequence
  Nucleoprotein (A/California/07/2009(H1N1)) forward primer
ccagatcagtgtgcagccta

SEQ ID NO: 32 - DNA, 22 bp, Artificial Sequence
  Nucleoprotein (A/California/07/2009(H1N1)) reverse primer
ggctttgcactttccatcattc

SEQ ID NO: 33 - DNA, 22 bp, Artificial Sequence
  Interferon beta (Mouse) forward primer
ttacactcgctttgccatccaa

SEQ ID NO: 34 - DNA, 22 bp, Artificial Sequence
  Interferon beta (Mouse) reverse primer
tcccacgtcaatctttcctctt